European Patent Application EP 4 430 948 A1, published September 18, 2024. Title: Strobilurin degrading bacteria and compositions. Applicant: Multikraft Produktions- und Handels GmbH. The sequence listing filed with the application follows.

SEQUENCE LISTING (9 sequences)

SEQ ID NO: 1 - RNA, 1458 nt, Bacillus sp. strain MK101
  source 1..1458: mol_type = rRNA
ttcggcggctggctcctaaaaggttacctcaccgacttcgggtgttacaaactctcgtggtgtgacgggcggtgtgtacaaggcccgggaacgtattcaccgcggcatgctgatccgcgattactagcgattccagcttcacgcagtcgagttgcagactgcgatccgaactgagaacagatttgtgggattggcttaacctcgcggtttcgctgccctttgttctgtccattgtagcacgtgtgtagcccaggtcataaggggcatgatgatttgacgtcatccccaccttcctccggtttgtcaccggcagtcaccttagagtgcccaactgaatgctggcaactaagatcaagggttgcgctcgttgcgggacttaacccaacatctcacgacacgagctgacgacaaccatgcaccacctgtcactctgcccccgaaggggacgtcctatctctaggattgtcagaggatgtcaagacctggtaaggttcttcgcgttgcttcgaattaaaccacatgctccaccgcttgtgcgggcccccgtcaattcctttgagtttcagtcttgcgaccgtactccccaggcggagtgcttaatgcgttagctgcagcactaaggggcggaaaccccctaacacttagcactcatcgtttacggcgtggactaccagggtatctaatcctgttcgctccccacgctttcgctcctcagcgtcagttacagaccagagagtcgccttcgccactggtgttcctccacatctctacgcatttcaccgctacacgtggaattccactctcctcttctgcactcaagttccccagtttccaatgaccctccccggttgagccgggggctttcacatcagacttaagaaaccgcctgcgagccctttacgcccaataattccggacaacgcttgccacctacgtattaccgcggctgctggcacgtagttagccgtggctttctggttaggtaccgtcaaggtaccgccctattcgaacggtacttgttcttccctaacaacagagctttacgatccgaaaaccttcatcactcacgcggcgttgctccgtcagactttcgtccattgcggaagattccctactgctgcctcccgtaggagtctgggccgtgtctcagtcccagtgtggccgatcaccctctcaggtcggctacgcatcgttgccttggtgagccgttacctcaccaactagctaatgcgccgcgggtccatctgtaagtggtagccgaagccaccttttatgtttgaaccatgcggttcaaacaaccatccggtattagccccggtttcccggagttatcccagtcttacaggcaggttacccacgtgttactcacccgtccgccgctaacatcagggagcaagctcccatctgtccgctcgacttgcatgtattaggcacgccgccagcgttcgtcctgagcag

SEQ ID NO: 2 - RNA, 830 nt, Rhodococcus sp. strain MK144
  source 1..830: mol_type = rRNA
gcgcttaatgcgttagctacggcacagatcccgtggaaggaacccacacctagcgcccaccgtttacggcgtggactaccagggtatctaatcctgtttgctacccacgctttcgttcctcagcgtcagttgtttcccagagacccgccttcgccaccggtgttcctcctgatatctgcgcatttcaccgctacaccaggaattccagtctcccctgaaacactcaagtctgcccgtatcgcctgcaagcccgaagttgagccccgggttttcacaaacgacgcgacaaaccgcctacgaactctttacgcccagtaattccggacaacgctcgcaccctacgtattaccgcggctgctggcacgtagttagccggtgcttcttctgcaggtaccgtcactcacgcttcgtccctgctgaaagaggtttacaacccgaaggccttcatccctcacgcggcgtcgctgcatcaggcttccgcccattgtgcaatattccccactgctgcctcccgtaggagtctgggccgtgtctcagtcccagtgtggccggtcaccctctcaggtcggctacccgtcgtcgccttggtaggccattaccccaccaacaagctgataggccgcgggcccatcctgcaccgataaatctttccaccacaacacatgcatgctgtggtcatatccggtattagacccagtttcccaagcttatcccagagtgcagggcagatcacccacgtgttactcacccgttcgccgctcgtgtaccccgaaaggccttaccgctcgacttgcatgtgttaagcacgccgccagcgttcgtcctgagca

SEQ ID NO: 3 - RNA, 1483 nt, Pseudomonas sp. strain MK113
  source 1..1483: mol_type = rRNA
ccgtcctcccgaaggttagactagctacttctggtgcaacccactcccatggtgtgacgggcggtgtgtacaaggcccgggaacgtattcaccgcgacattctgattcgcgattactagcgattccgacttcacgcagtcgagttgcagactgcgatccggactacgatcggttttgtgagattagctccacctcgcggcttggcaaccctctgtaccgaccattgtagcacgtgtgtagcccaggccgtaagggccatgatgacttgacgtcatccccaccttcctccggtttgtcaccggcagtctccttagagtgcccaccataacgtgctggtaactaaggacaagggttgcgctcgttacgggacttaacccaacatctcacgacacgagctgacgacagccatgcagcacctgtgtcagagttcccgaaggcaccaatccatctctggaaagttctctgcatgtcaaggcctggtaaggttcttcgcgttgcttcgaattaaaccacatgctccaccgcttgtgcgggcccccgtcaattcatttgagttttaaccttgcggccgtactccccaggcggtcaacttaatgcgttagctgcgccactaaaatctcaaggattccaacggctagttgacatcgtttacggcgtggactaccagggtatctaatcctgtttgctccccacgctttcgcacctcagtgtcagtatcagtccaggtggtcgccttcgccactggtgttccttcctatatctacgcatttcaccgctacacaggaaattccaccaccctctaccgtactctagcttgccagttttggatgcagttcccaggttgagcccggggctttcacatccaacttaacaaaccacctacgcgcgctttacgcccagtaattccgattaacgcttgcaccctctgtattaccgcggctgctggcacagagttagccggtgcttattctgtcggtaacgtcaaaacagcaaggtattcgcttactgcccttcctcccaacttaaagtgctttacaatccgaagaccttcttcacacacgcggcatggctggatcaggctttcgcccattgtccaatattccccactgctgcctcccgtaggagtctggaccgtgtctcagttccagtgtgactgatcatcctctcagaccagttacggatcgtcgccttggtgagccattaccccaccaactagctaatccgacctaggctcatctgatagcgcaaggcccgaaggtcccctgctttctcccgtaggacgtatgcggtattagcgttcctttcgaaacgttgtcccccactaccaggcagattcctaggcattactcacccgtccgccgctgaatcgaagagcaagctcttctcatccgctcgacttgcatgtgttaggcctgccgccagcgttcaatctgagcctcgacttgcatgtgtaaggcatgccgccagcgttcaatctgagcag

SEQ ID NO: 4 - DNA, 18 bp, synthetic construct
  source 1..18: mol_type = other DNA
ggctgcttctaagccaac

SEQ ID NO: 5 - DNA, 20 bp, synthetic construct
  source 1..20: mol_type = other DNA
tgcggctggatcacctcctt

SEQ ID NO: 6 - DNA, 20 bp, synthetic construct
  source 1..20: mol_type = other DNA
agagtttgatcctggctcag

SEQ ID NO: 7 - DNA, 20 bp, synthetic construct
  source 1..20: mol_type = other DNA
aaggaggtgatccagccgca

SEQ ID NO: 8 - DNA, 20 bp, synthetic construct
  source 1..20: mol_type = other DNA
ccgtcaattcctttgagttt

SEQ ID NO: 9 - DNA, 19 bp, synthetic construct
  source 1..19: mol_type = other DNA
ggttaccttgttacgactt